European Patent Specification EP 4 011 915 B1, published October 11, 2023. Title: Methods for Treating or Preventing Asthma by Administering an IL-4R Antagonist. Applicant: Sanofi Biotechnology et al. The sequence listing filed with the application follows.

SEQUENCE LISTING (275 sequences)

SEQ ID NO: 1 - DNA, 351 bp, Artificial Sequence
  Synthetic
caggtgcagctggtggagtctgggggaggcgtggtccagcctgggaggtccctgagactctcctgtgcagcctctggattcaccttccgctcttatggcatgcactgggtccgccaggctccaggcaaggggctggagtgggtggcggtcatatcatatgatggaagtaataaatattatatagactccgtgaagggccgattcaccatctccagagacaattccaagaacacgctgaatctgcaaatgaacagcctgagacttgaggacacggctgtatattactgtgcgaaagaggggagggggggatttgactactggggccagggaatcccggtcaccgtctcctca

SEQ ID NO: 2 - protein, 117 aa, Artificial Sequence
  Synthetic
QVQLVESGGGVVQPGRSLRLSCAASGFTFRSYGMHWVRQAPGKGLEWVAVISYDGSNKYYIDSVKGRFTISRDNSKNTLNLQMNSLRLEDTAVYYCAKEGRGGFDYWGQGIPVTVSS

SEQ ID NO: 3 - DNA, 24 bp, Artificial Sequence
  Synthetic
ggattcaccttccgctcttatggc

SEQ ID NO: 4 - protein, 8 aa, Artificial Sequence
  Synthetic
GFTFRSYG

SEQ ID NO: 5 - DNA, 24 bp, Artificial Sequence
  Synthetic
atatcatatgatggaagtaataaa

SEQ ID NO: 6 - protein, 8 aa, Artificial Sequence
  Synthetic
ISYDGSNK

SEQ ID NO: 7 - DNA, 30 bp, Artificial Sequence
  Synthetic
gcgaaagaggggagggggggatttgactac

SEQ ID NO: 8 - protein, 10 aa, Artificial Sequence
  Synthetic
AKEGRGGFDY

SEQ ID NO: 9 - DNA, 324 bp, Artificial Sequence
  Synthetic
gacatccagatgacccagtctccatcctcactgtctgcatctgtaggagacagagtcaccatcacttgtcgggcgagtcaggtcataaacaattatttagcctggtttcagcagaaaccagggaaagtccctaagtccctgatccatgctgcatccagtttacaaagtggggtcccatcaaagttcagcggcagtggatctgggacagatttcactctcaccatcagcagcctgcagcctgaagattttgcaacttattactgccaacagtataatagtcacccgtggacgttcggccaagggaccaaggtggaaatcaaacga

SEQ ID NO: 10 - protein, 108 aa, Artificial Sequence
  Synthetic
DIQMTQSPSSLSASVGDRVTITCRASQVINNYLAWFQQKPGKVPKSLIHAASSLQSGVPSKFSGSGSGTDFTLTISSLQPEDFATYYCQQYNSHPWTFGQGTKVEIKR

SEQ ID NO: 11 - DNA, 18 bp, Artificial Sequence
  Synthetic
caggtcataaacaattat

SEQ ID NO: 12 - protein, 6 aa, Artificial Sequence
  Synthetic
QVINNY

SEQ ID NO: 13 - DNA, 9 bp, Artificial Sequence
  Synthetic
gctgcatcc

SEQ ID NO: 14 - protein, 3 aa, Artificial Sequence
  Synthetic
AAS

SEQ ID NO: 15 - DNA, 27 bp, Artificial Sequence
  Synthetic
caacagtataatagtcacccgtggacg

SEQ ID NO: 16 - protein, 9 aa, Artificial Sequence
  Synthetic
QQYNSHPWT

SEQ ID NO: 17 - DNA, 351 bp, Artificial Sequence
  Synthetic
caggtgcagctggtggagtctgggggaggcgtggtccagcctgggaggtccctgagactctcctgtgcagcctctggattcaccttccgctcttatggcatgcactgggtccgccaggctccaggcaaggggctggagtgggtggcggtcatatcatatgatggaagtaataaatattatatagactccgtgaagggccgattcaccatctccagagacaattccaagaacacgctgaatctgcaaatgaacagcctgagacttgaggacacggctgtatattactgtgcgaaagaggggagggggggatttgactactggggccagggaaccctggtcaccgtctcctca

SEQ ID NO: 18 - protein, 117 aa, Artificial Sequence
  Synthetic
QVQLVESGGGVVQPGRSLRLSCAASGFTFRSYGMHWVRQAPGKGLEWVAVISYDGSNKYYIDSVKGRFTISRDNSKNTLNLQMNSLRLEDTAVYYCAKEGRGGFDYWGQGTLVTVSS

SEQ ID NO: 19 - DNA, 321 bp, Artificial Sequence
  Synthetic
gacatccagatgacccagtctccatcctcactgtctgcatctgtaggagacagagtcaccatcacttgtcgggcgagtcaggtcataaacaattatttagcctggtttcagcagaaaccagggaaagtccctaagtccctgatccatgctgcatccagtttacaaagtggggtcccatcaaagttcagcggcagtggatctgggacagatttcactctcaccatcagcagcctgcagcctgaagattttgcaacttattactgccaacagtataatagtcacccgtggacgttcggccaagggaccaaggtggaaatcaaa

SEQ ID NO: 20 - protein, 107 aa, Artificial Sequence
  Synthetic
DIQMTQSPSSLSASVGDRVTITCRASQVINNYLAWFQQKPGKVPKSLIHAASSLQSGVPSKFSGSGSGTDFTLTISSLQPEDFATYYCQQYNSHPWTFGQGTKVEIK

SEQ ID NO: 21 - DNA, 351 bp, Artificial Sequence
  Synthetic
caggtgcagctggtggagtctgggggaggcgtggtccagcctgggaggtccctgagactctcctgtgcagcctctggattcaccttccgctcttatggcatgcactgggtccgccaggctccaggcaaggggctggagtgggtggcagttatatcatatgatggaagtaataaatactatgcagactccgtgaagggccgattcaccatctccagagacaattccaagaacacgctgtatctgcaaatgaacagcctgagagctgaggacacggctgtgtattactgtgcgaaagaggggagggggggatttgactactggggccagggaaccctggtcaccgtctcctca

SEQ ID NO: 22 - protein, 117 aa, Artificial Sequence
  Synthetic
QVQLVESGGGVVQPGRSLRLSCAASGFTFRSYGMHWVRQAPGKGLEWVAVISYDGSNKYYADSVKGRFTISRDNSKNTLYLQMNSLRAEDTAVYYCAKEGRGGFDYWGQGTLVTVSS

SEQ ID NO: 23 - DNA, 322 bp, Artificial Sequence
  Synthetic
gacatccagatgacccagtctccatcctcactgtctgcatctgtaggagacagagtcaccatcacttgtcgggcgagtcaggtcataaacaattatttagcctggtttcagcagaaaccagggaaagcccctaagtccctgatctatgctgcatccagtttgcaaagtggggtcccatcaaggttcagcggcagtggatctgggacagatttcactctcaccatcagcagcctgcagcctgaagattttgcaacttattactgccaacagtataatagtcacccgtggacgttcggccaagggaccaaggtggaaatcaaac

SEQ ID NO: 24 - protein, 107 aa, Artificial Sequence
  Synthetic
DIQMTQSPSSLSASVGDRVTITCRASQVINNYLAWFQQKPGKAPKSLIYAASSLQSGVPSRFSGSGSGTDFTLTISSLQPEDFATYYCQQYNSHPWTFGQGTKVEIK

SEQ ID NO: 25 - DNA, 351 bp, Artificial Sequence
  Synthetic
caggtgcagctggtggagtctgggggaggcgtggtccagcctgggaggtccctgagactctcctgtgcagcctctggattcaccttcagaagctatggcatacactgggtccgccaggctccaggcaaggggctggagtgggtggcagttatatcatatgatggaagtaataaatactatgcagactccgtgaagggccgattcaccatctccagagacaattccaagaacacactgtatctgcaaatgaacagcctgataactgaggacacggctgtgtattattgtgtgaaagaggggaggggggggtttgactactggggccagggaaccacggtcaccgtctcctca

SEQ ID NO: 26 - protein, 117 aa, Artificial Sequence
  Synthetic
QVQLVESGGGVVQPGRSLRLSCAASGFTFRSYGIHWVRQAPGKGLEWVAVISYDGSNKYYADSVKGRFTISRDNSKNTLYLQMNSLITEDTAVYYCVKEGRGGFDYWGQGTTVTVSS

SEQ ID NO: 27 - DNA, 24 bp, Artificial Sequence
  Synthetic
ggattcaccttcagaagctatggc

SEQ ID NO: 28 - protein, 8 aa, Artificial Sequence
  Synthetic
GFTFRSYG

SEQ ID NO: 29 - DNA, 24 bp, Artificial Sequence
  Synthetic
atatcatatgatggaagtaataaa

SEQ ID NO: 30 - protein, 8 aa, Artificial Sequence
  Synthetic
ISYDGSNK

SEQ ID NO: 31 - DNA, 30 bp, Artificial Sequence
  Synthetic
gtgaaagaggggaggggggggtttgactac

SEQ ID NO: 32 - protein, 10 aa, Artificial Sequence
  Synthetic
VKEGRGGFDY

SEQ ID NO: 33 - DNA, 324 bp, Artificial Sequence
  Synthetic
gacatccagatgacccagtctccatcctcactgtctgcatctgtaggagacagagtcaccatcacttgtcgggcgagtcaggtcattaataattatttagcctggtttcagcagaaaccagggaaagtccctaagtccctgatccatgctgcatccagtttgcaaagaggggtcccatcaaagttcagcggcagtggatctgggacagatttcactctcaccatcaacagcctgcagcctgaagattttgcaacttattactgccaacaatataatagttacccgtggacgttcggccaagggaccaaggtggaaatcaaacga

SEQ ID NO: 34 - protein, 108 aa, Artificial Sequence
  Synthetic
DIQMTQSPSSLSASVGDRVTITCRASQVINNYLAWFQQKPGKVPKSLIHAASSLQRGVPSKFSGSGSGTDFTLTINSLQPEDFATYYCQQYNSYPWTFGQGTKVEIKR

SEQ ID NO: 35 - DNA, 18 bp, Artificial Sequence
  Synthetic
caggtcattaataattat

SEQ ID NO: 36 - protein, 6 aa, Artificial Sequence
  Synthetic
QVINNY

SEQ ID NO: 37 - DNA, 9 bp, Artificial Sequence
  Synthetic
gctgcatcc

SEQ ID NO: 38 - protein, 3 aa, Artificial Sequence
  Synthetic
AAS

SEQ ID NO: 39 - DNA, 27 bp, Artificial Sequence
  Synthetic
caacaatataatagttacccgtggacg

SEQ ID NO: 40 - protein, 9 aa, Artificial Sequence
  Synthetic
QQYNSYPWT

SEQ ID NO: 41 - DNA, 351 bp, Artificial Sequence
  Synthetic
caggtgcagctggtggagtctgggggaggcgtggtccagcctgggaggtccctgagactctcctgtgcagcctctggattcaccttcagaagctatggcatacactgggtccgccaggctccaggcaaggggctggagtgggtggcagttatatcatatgatggaagtaataaatactatgcagactccgtgaagggccgattcaccatctccagagacaattccaagaacacactgtatctgcaaatgaacagcctgataactgaggacacggctgtgtattattgtgtgaaagaggggaggggggggtttgactactggggccagggaaccctggtcaccgtctcctca

SEQ ID NO: 42 - protein, 117 aa, Artificial Sequence
  Synthetic
QVQLVESGGGVVQPGRSLRLSCAASGFTFRSYGIHWVRQAPGKGLEWVAVISYDGSNKYYADSVKGRFTISRDNSKNTLYLQMNSLITEDTAVYYCVKEGRGGFDYWGQGTLVTVSS

SEQ ID NO: 43 - DNA, 321 bp, Artificial Sequence
  Synthetic
gacatccagatgacccagtctccatcctcactgtctgcatctgtaggagacagagtcaccatcacttgtcgggcgagtcaggtcattaataattatttagcctggtttcagcagaaaccagggaaagtccctaagtccctgatccatgctgcatccagtttgcaaagaggggtcccatcaaagttcagcggcagtggatctgggacagatttcactctcaccatcaacagcctgcagcctgaagattttgcaacttattactgccaacaatataatagttacccgtggacgttcggccaagggaccaaggtggaaatcaaa

SEQ ID NO: 44 - protein, 107 aa, Artificial Sequence
  Synthetic
DIQMTQSPSSLSASVGDRVTITCRASQVINNYLAWFQQKPGKVPKSLIHAASSLQRGVPSKFSGSGSGTDFTLTINSLQPEDFATYYCQQYNSYPWTFGQGTKVEIK

SEQ ID NO: 45 - DNA, 351 bp, Artificial Sequence
  Synthetic
caggtgcagctggtggagtctgggggaggcgtggtccagcctgggaggtccctgagactctcctgtgcagcctctggattcaccttcagaagctatggcatgcactgggtccgccaggctccaggcaaggggctggagtgggtggcagttatatcatatgatggaagtaataaatactatgcagactccgtgaagggccgattcaccatctccagagacaattccaagaacacgctgtatctgcaaatgaacagcctgagagctgaggacacggctgtgtattactgtgtgaaagaggggaggggggggtttgactactggggccagggaaccctggtcaccgtctcctca

SEQ ID NO: 46 - protein, 117 aa, Artificial Sequence
  Synthetic
QVQLVESGGGVVQPGRSLRLSCAASGFTFRSYGMHWVRQAPGKGLEWVAVISYDGSNKYYADSVKGRFTISRDNSKNTLYLQMNSLRAEDTAVYYCVKEGRGGFDYWGQGTLVTVSS

SEQ ID NO: 47 - DNA, 322 bp, Artificial Sequence
  Synthetic
gacatccagatgacccagtctccatcctcactgtctgcatctgtaggagacagagtcaccatcacttgtcgggcgagtcaggtcattaataattatttagcctggtttcagcagaaaccagggaaagcccctaagtccctgatctatgctgcatccagtttgcaaagtggggtcccatcaaggttcagcggcagtggatctgggacagatttcactctcaccatcagcagcctgcagcctgaagattttgcaacttattactgccaacaatataatagttacccgtggacgttcggccaagggaccaaggtggaaatcaaac

SEQ ID NO: 48 - protein, 107 aa, Artificial Sequence
  Synthetic
DIQMTQSPSSLSASVGDRVTITCRASQVINNYLAWFQQKPGKAPKSLIYAASSLQSGVPSRFSGSGSGTDFTLTISSLQPEDFATYYCQQYNSYPWTFGQGTKVEIK

SEQ ID NO: 49 - DNA, 375 bp, Artificial Sequence
  Synthetic
caggtgcagctggtggagtctgggggaggcttggaacagccgggggggtccttgagactctcctgtgcaggctctggattcacgtttagagactatgccatgacctgggtccgccaggctccagggaaggggctggagtgggtcgcatcgattagtggttccggtggtaacacatacttcgcagactccgtgaagggccggttcaccatctccagagacaattccaagaacacgctgtatctgcaaatgaacagcctgagagccgaggacacggccgtatattactgtgcgaaagatcgactctctataacaattcgcccacgctattatggtttggacgtctggggccaagggtccacggtcaccgtctcctca

SEQ ID NO: 50 - protein, 125 aa, Artificial Sequence
  Synthetic
QVQLVESGGGLEQPGGSLRLSCAGSGFTFRDYAMTWVRQAPGKGLEWVASISGSGGNTYFADSVKGRFTISRDNSKNTLYLQMNSLRAEDTAVYYCAKDRLSITIRPRYYGLDVWGQGSTVTVSS

SEQ ID NO: 51 - DNA, 24 bp, Artificial Sequence
  Synthetic
ggattcacgtttagagactatgcc

SEQ ID NO: 52 - protein, 8 aa, Artificial Sequence
  Synthetic
GFTFRDYA

SEQ ID NO: 53 - DNA, 24 bp, Artificial Sequence
  Synthetic
attagtggttccggtggtaacaca

SEQ ID NO: 54 - protein, 8 aa, Artificial Sequence
  Synthetic
ISGSGGNT

SEQ ID NO: 55 - DNA, 54 bp, Artificial Sequence
  Synthetic
gcgaaagatcgactctctataacaattcgcccacgctattatggtttggacgtc

SEQ ID NO: 56 - protein, 18 aa, Artificial Sequence
  Synthetic
AKDRLSITIRPRYYGLDV

SEQ ID NO: 57 - DNA, 324 bp, Artificial Sequence
  Synthetic
gacatccagatgacccagtctccatcctcactgtctgcatctgttggagacagagtcaccatcacttgtcgggcgagtcaggccattaacaatcatttagcctggtttcagcagaaaccagggaaagcccctaagtccctgatctttgctgtatccagtttgcaaagtggggtcccatcaaagttcagcggcagtggatctgggacagacttcactctcaccatcagcagcctgcagcctgaagattttgcaacttattactgccaacagtataatagttacccgtggacgttcggccaagggaccaaggtggaaatcaaacga

SEQ ID NO: 58 - protein, 108 aa, Artificial Sequence
  Synthetic
DIQMTQSPSSLSASVGDRVTITCRASQAINNHLAWFQQKPGKAPKSLIFAVSSLQSGVPSKFSGSGSGTDFTLTISSLQPEDFATYYCQQYNSYPWTFGQGTKVEIKR

SEQ ID NO: 59 - DNA, 18 bp, Artificial Sequence
  Synthetic
caggccattaacaatcat

SEQ ID NO: 60 - protein, 6 aa, Artificial Sequence
  Synthetic
QAINNH

SEQ ID NO: 61 - DNA, 9 bp, Artificial Sequence
  Synthetic
gctgtatcc

SEQ ID NO: 62 - protein, 3 aa, Artificial Sequence
  Synthetic
AVS

SEQ ID NO: 63 - DNA, 27 bp, Artificial Sequence
  Synthetic
caacagtataatagttacccgtggacg

SEQ ID NO: 64 - protein, 9 aa, Artificial Sequence
  Synthetic
QQYNSYPWT

SEQ ID NO: 65 - DNA, 372 bp, Artificial Sequence
  Synthetic
gaggtgcagctggtggagtctgggggaggcttggaacagccgggggggtccttgagactctcctgtgcaggctctggattcacgtttagagactatgccatgacctgggtccgccaggctccagggaaggggctggagtgggtcgcatcgattagtggttccggtggtaacacatacttcgcagactccgtgaagggccggttcaccatctccagagacaattccaagaacacgctgtatctgcaaatgaacagcctgagagccgaggacacggccgtatattactgtgcgaaagatcgactctctataacaattcgcccacgctattatggtttggacgtctggggccaagggaccacggtcaccgtctcc

SEQ ID NO: 66 - protein, 124 aa, Artificial Sequence
  Synthetic
EVQLVESGGGLEQPGGSLRLSCAGSGFTFRDYAMTWVRQAPGKGLEWVASISGSGGNTYFADSVKGRFTISRDNSKNTLYLQMNSLRAEDTAVYYCAKDRLSITIRPRYYGLDVWGQGTTVTVS

SEQ ID NO: 67 - DNA, 321 bp, Artificial Sequence
  Synthetic
gacatccagatgacccagtctccatcctcactgtctgcatctgttggagacagagtcaccatcacttgtcgggcgagtcaggccattaacaatcatttagcctggtttcagcagaaaccagggaaagcccctaagtccctgatctttgctgtatccagtttgcaaagtggggtcccatcaaagttcagcggcagtggatctgggacagacttcactctcaccatcagcagcctgcagcctgaagattttgcaacttattactgccaacagtataatagttacccgtggacgttcggccaagggaccaaggtggaaatcaaa

SEQ ID NO: 68 - protein, 107 aa, Artificial Sequence
  Synthetic
DIQMTQSPSSLSASVGDRVTITCRASQAINNHLAWFQQKPGKAPKSLIFAVSSLQSGVPSKFSGSGSGTDFTLTISSLQPEDFATYYCQQYNSYPWTFGQGTKVEIK

SEQ ID NO: 69 - DNA, 373 bp, Artificial Sequence
  Synthetic
gaggtgcagctggtggagtctgggggaggcttggtacagcctggggggtccctgagactctcctgtgcagcctctggattcacgtttagagactatgccatgagctgggtccgccaggctccagggaaggggctggagtgggtctcagctattagtggttccggtggtaacacatactacgcagactccgtgaagggccggttcaccatctccagagacaattccaagaacacgctgtatctgcaaatgaacagcctgagagccgaggacacggccgtatattactgtgcgaaagatcgactctctataacaattcgcccacgctattatggtttggacgtctggggccaagggaccacggtcaccgtctcct

SEQ ID NO: 70 - protein, 124 aa, Artificial Sequence
  Synthetic
EVQLVESGGGLVQPGGSLRLSCAASGFTFRDYAMSWVRQAPGKGLEWVSAISGSGGNTYYADSVKGRFTISRDNSKNTLYLQMNSLRAEDTAVYYCAKDRLSITIRPRYYGLDVWGQGTTVTVS

SEQ ID NO: 71 - DNA, 322 bp, Artificial Sequence
  Synthetic
gacatccagatgacccagtctccatcctcactgtctgcatctgtaggagacagagtcaccatcacttgtcgggcgagtcaggccattaacaatcatttagcctggtttcagcagaaaccagggaaagcccctaagtccctgatctatgctgtatccagtttgcaaagtggggtcccatcaaggttcagcggcagtggatctgggacagatttcactctcaccatcagcagcctgcagcctgaagattttgcaacttattactgccaacagtataatagttacccgtggacgttcggccaagggaccaaggtggaaatcaaac

SEQ ID NO: 72 - protein, 107 aa, Artificial Sequence
  Synthetic
DIQMTQSPSSLSASVGDRVTITCRASQAINNHLAWFQQKPGKAPKSLIYAVSSLQSGVPSRFSGSGSGTDFTLTISSLQPEDFATYYCQQYNSYPWTFGQGTKVEIK

SEQ ID NO: 73 - DNA, 375 bp, Artificial Sequence; identical to SEQ ID NO: 49
  Synthetic

SEQ ID NO: 74 - protein, 125 aa, Artificial Sequence; identical to SEQ ID NO: 50
  Synthetic

SEQ ID NO: 75 - DNA, 24 bp, Artificial Sequence
  Synthetic
ggattcacgtttagagactatgcc

SEQ ID NO: 76 - protein, 8 aa, Artificial Sequence
  Synthetic
GFTFRDYA

SEQ ID NO: 77 - DNA, 24 bp, Artificial Sequence
  Synthetic
attagtggttccggtggtaacaca

SEQ ID NO: 78 - protein, 8 aa, Artificial Sequence
  Synthetic
ISGSGGNT

SEQ ID NO: 79 - DNA, 54 bp, Artificial Sequence; identical to SEQ ID NO: 55
  Synthetic

SEQ ID NO: 80 - protein, 18 aa, Artificial Sequence
  Synthetic
AKDRLSITIRPRYYGLDV

SEQ ID NO: 81 - DNA, 339 bp, Artificial Sequence
  Synthetic
gaaatagtgttgacgcagtctccactctccctgcccgtcacccctggagagccggcctccatctcctgcaggtctagtcagagcctcctgtatagtattggatacaactatttggattggtacctgcagaagtcagggcagtctccacagctccttatctatttgggttctaatcgggcctccggggtccctgacaggttcagtggcagtggatcaggcacagattttacactgaaaatcagcagagtggaggctgaggatgttgggttttattactgcatgcaagctctacaaactccgtacacttttggcccggggaccaagctggagatcaaacga

SEQ ID NO: 82 - protein, 113 aa, Artificial Sequence
  Synthetic
EIVLTQSPLSLPVTPGEPASISCRSSQSLLYSIGYNYLDWYLQKSGQSPQLLIYLGSNRASGVPDRFSGSGSGTDFTLKISRVEAEDVGFYYCMQALQTPYTFGPGTKLEIKR

SEQ ID NO: 83 - DNA, 33 bp, Artificial Sequence
  Synthetic
cagagcctcctgtatagtattggatacaactat

SEQ ID NO: 84 - protein, 11 aa, Artificial Sequence
  Synthetic
QSLLYSIGYNY

SEQ ID NO: 85 - DNA, 9 bp, Artificial Sequence
  Synthetic
ttgggttct

SEQ ID NO: 86 - protein, 3 aa, Artificial Sequence
  Synthetic
LGS

SEQ ID NO: 87 - DNA, 27 bp, Artificial Sequence
  Synthetic
atgcaagctctacaaactccgtacact

SEQ ID NO: 88 - protein, 9 aa, Artificial Sequence
  Synthetic
MQALQTPYT

SEQ ID NO: 89 - DNA, 372 bp, Artificial Sequence; identical to SEQ ID NO: 65
  Synthetic

SEQ ID NO: 90 - protein, 124 aa, Artificial Sequence; identical to SEQ ID NO: 66
  Synthetic

SEQ ID NO: 91 - DNA, 336 bp, Artificial Sequence
  Synthetic
gatattgtgatgactcagtctccactctccctgcccgtcacccctggagagccggcctccatctcctgcaggtctagtcagagcctcctgtatagtattggatacaactatttggattggtacctgcagaagtcagggcagtctccacagctccttatctatttgggttctaatcgggcctccggggtccctgacaggttcagtggcagtggatcaggcacagattttacactgaaaatcagcagagtggaggctgaggatgttgggttttattactgcatgcaagctctacaaactccgtacacttttggcccggggaccaagctggagatcaaa

SEQ ID NO: 92 - protein, 112 aa, Artificial Sequence
  Synthetic
DIVMTQSPLSLPVTPGEPASISCRSSQSLLYSIGYNYLDWYLQKSGQSPQLLIYLGSNRASGVPDRFSGSGSGTDFTLKISRVEAEDVGFYYCMQALQTPYTFGPGTKLEIK

SEQ ID NO: 93 - DNA, 373 bp, Artificial Sequence; identical to SEQ ID NO: 69
  Synthetic

SEQ ID NO: 94 - protein, 124 aa, Artificial Sequence; identical to SEQ ID NO: 70
  Synthetic

SEQ ID NO: 95 - DNA, 337 bp, Artificial Sequence
  Synthetic
gatattgtgatgactcagtctccactctccctgcccgtcacccctggagagccggcctccatctcctgcaggtctagtcagagcctcctgtatagtattggatacaactatttggattggtacctgcagaagccagggcagtctccacagctcctgatctatttgggttctaatcgggcctccggggtccctgacaggttcagtggcagtggatcaggcacagattttacactgaaaatcagcagagtggaggctgaggatgttggggtttattactgcatgcaagctctacaaactccgtacacttttggccaggggaccaagctggagatcaaac

SEQ ID NO: 96 - protein, 112 aa, Artificial Sequence
  Synthetic
DIVMTQSPLSLPVTPGEPASISCRSSQSLLYSIGYNYLDWYLQKPGQSPQLLIYLGSNRASGVPDRFSGSGSGTDFTLKISRVEAEDVGVYYCMQALQTPYTFGQGTKLEIK

SEQ ID NO: 97 - DNA, 375 bp, Artificial Sequence
  Synthetic
caggtgcagctggtggagtctgagggactcttggaacagcctggggggtccctgagactctcctgtgcagcctctggattcaactttagagactttgccatgacctgggtccgccaggctccagggaaggggctggagtgggtctcatctattagtggtagtggtagtaatacatactacgcagactccgtgaagggccggttcaccatctccagagacaattccaaccacacgctgtatctgcgaatgaacagcctgagagccgaagacacggccgtgtattactgtgcgaaagatcgactctctataacaattcgcccacgctattacggtctggacgtctggggccaagggtccacggtcaccgtctcctca

SEQ ID NO: 98 - protein, 125 aa, Artificial Sequence
  Synthetic
QVQLVESEGLLEQPGGSLRLSCAASGFNFRDFAMTWVRQAPGKGLEWVSSISGSGSNTYYADSVKGRFTISRDNSNHTLYLRMNSLRAEDTAVYYCAKDRLSITIRPRYYGLDVWGQGSTVTVSS

SEQ ID NO: 99 - DNA, 24 bp, Artificial Sequence
  Synthetic
ggattcaactttagagactttgcc

SEQ ID NO: 100 - protein, 8 aa, Artificial Sequence
  Synthetic
GFNFRDFA

SEQ ID NO: 101 - DNA, 24 bp, Artificial Sequence
  Synthetic
attagtggtagtggtagtaataca

SEQ ID NO: 102 - protein, 8 aa, Artificial Sequence
  Synthetic
ISGSGSNT

SEQ ID NO: 103 - DNA, 54 bp, Artificial Sequence
  Synthetic
gcgaaagatcgactctctataacaattcgcccacgctattacggtctggacgtc

SEQ ID NO: 104 - protein, 18 aa, Artificial Sequence
  Synthetic
AKDRLSITIRPRYYGLDV

SEQ ID NO: 105 - DNA, 324 bp, Artificial Sequence
  Synthetic
gacatccagatgacccagtctccatcctccctgtctgcatctgtaggagacagagtcaccatcacttgccgggcgagtcaggacattagcaattattttgcctggtatcagcagaagccagggaaagttcctaagctcctgatctttgctgcatccactttgcatccaggggtcccatctcggttcagtggcagtggatctgggacagatttcactctcaccattcgcagcctgcagcctgaagatgttgcaacttattactgtcaaaaatatgacagtgccccgtacacttttggccaggggaccaaggtggaaatcaaacga

SEQ ID NO: 106 - protein, 108 aa, Artificial Sequence
  Synthetic
DIQMTQSPSSLSASVGDRVTITCRASQDISNYFAWYQQKPGKVPKLLIFAASTLHPGVPSRFSGSGSGTDFTLTIRSLQPEDVATYYCQKYDSAPYTFGQGTKVEIKR

SEQ ID NO: 107 - DNA, 18 bp, Artificial Sequence
  Synthetic
caggacattagcaattat

SEQ ID NO: 108 - protein, 6 aa, Artificial Sequence
  Synthetic
QDISNY

SEQ ID NO: 109 - DNA, 9 bp, Artificial Sequence
  Synthetic
gctgcatcc

SEQ ID NO: 110 - protein, 3 aa, Artificial Sequence
  Synthetic
AAS

SEQ ID NO: 111 - DNA, 27 bp, Artificial Sequence
  Synthetic
caaaaatatgacagtgccccgtacact

SEQ ID NO: 112 - protein, 9 aa, Artificial Sequence
  Synthetic
QKYDSAPYT

SEQ ID NO: 113 - DNA, 372 bp, Artificial Sequence
  Synthetic
gaggtgcagctggtggagtctgagggactcttggaacagcctggggggtccctgagactctcctgtgcagcctctggattcaactttagagactttgccatgacctgggtccgccaggctccagggaaggggctggagtgggtctcatctattagtggtagtggtagtaatacatactacgcagactccgtgaagggccggttcaccatctccagagacaattccaaccacacgctgtatctgcgaatgaacagcctgagagccgaagacacggccgtgtattactgtgcgaaagatcgactctctataacaattcgcccacgctattacggtctggacgtctggggccaagggaccacggtcaccgtctcc

SEQ ID NO: 114 - protein, 124 aa, Artificial Sequence
  Synthetic
EVQLVESEGLLEQPGGSLRLSCAASGFNFRDFAMTWVRQAPGKGLEWVSSISGSGSNTYYADSVKGRFTISRDNSNHTLYLRMNSLRAEDTAVYYCAKDRLSITIRPRYYGLDVWGQGTTVTVS

SEQ ID NO: 115 - DNA, 321 bp, Artificial Sequence
  Synthetic
gacatccagatgacccagtctccatcctccctgtctgcatctgtaggagacagagtcaccatcacttgccgggcgagtcaggacattagcaattattttgcctggtatcagcagaagccagggaaagttcctaagctcctgatctttgctgcatccactttgcatccaggggtcccatctcggttcagtggcagtggatctgggacagatttcactctcaccattcgcagcctgcagcctgaagatgttgcaacttattactgtcaaaaatatgacagtgccccgtacacttttggccaggggaccaagctggagatcaaa

SEQ ID NO: 116 - protein, 107 aa, Artificial Sequence
  Synthetic
DIQMTQSPSSLSASVGDRVTITCRASQDISNYFAWYQQKPGKVPKLLIFAASTLHPGVPSRFSGSGSGTDFTLTIRSLQPEDVATYYCQKYDSAPYTFGQGTKLEIK

SEQ ID NO: 117 - DNA, 373 bp, Artificial Sequence
  Synthetic
gaggtgcagctggtggagtctgggggaggcttggtacagcctggggggtccctgagactctcctgtgcagcctctggattcaactttagagactttgccatgagctgggtccgccaggctccagggaaggggctggagtgggtctcagctattagtggtagtggtagtaatacatactacgcagactccgtgaagggccggttcaccatctccagagacaattccaagaacacgctgtatctgcaaatgaacagcctgagagccgaggacacggccgtatattactgtgcgaaagatcgactctctataacaattcgcccacgctattacggtctggacgtctggggccaagggaccacggtcaccgtctcct

SEQ ID NO: 118 - protein, 124 aa, Artificial Sequence
  Synthetic
EVQLVESGGGLVQPGGSLRLSCAASGFNFRDFAMSWVRQAPGKGLEWVSAISGSGSNTYYADSVKGRFTISRDNSKNTLYLQMNSLRAEDTAVYYCAKDRLSITIRPRYYGLDVWGQGTTVTVS

SEQ ID NO: 119 - DNA, 322 bp, Artificial Sequence
  Synthetic
gacatccagatgacccagtctccatcctccctgtctgcatctgtaggagacagagtcaccatcacttgccgggcgagtcaggacattagcaattatttagcctggtatcagcagaaaccagggaaagttcctaagctcctgatctatgctgcatccactttgcaatcaggggtcccatctcggttcagtggcagtggatctgggacagatttcactctcaccatcagcagcctgcagcctgaagatgttgcaacttattactgtcaaaaatatgacagtgccccgtacacttttggccaggggaccaagctggagatcaaac

SEQ ID NO: 120 - protein, 107 aa, Artificial Sequence
  Synthetic
DIQMTQSPSSLSASVGDRVTITCRASQDISNYLAWYQQKPGKVPKLLIYAASTLQSGVPSRFSGSGSGTDFTLTISSLQPEDVATYYCQKYDSAPYTFGQGTKLEIK

SEQ ID NO: 121 - DNA, 357 bp, Artificial Sequence
  Synthetic
caggtgcagctggtggagtctgggggaggcttggtacagcctggggggtccctgagactctcctgtgtagcttctggattcacccttaacaactttgtcatgaactgggtccgccaggttccagggaagggactggagtgggtctcttttattagtgctagtggtggtagtatatactacgcagactccgtgaagggccggttcaccatctccagagacacttccaagaacacattatatctgcaaatgaacagcctgagagccgacgacacggccgtctattactgtgcgaaatccccgtataactggaacccctttgactattggggccagggaaccacggtcaccgtctcctca

SEQ ID NO: 122 - protein, 119 aa, Artificial Sequence
  Synthetic
QVQLVESGGGLVQPGGSLRLSCVASGFTLNNFVMNWVRQVPGKGLEWVSFISASGGSIYYADSVKGRFTISRDTSKNTLYLQMNSLRADDTAVYYCAKSPYNWNPFDYWGQGTTVTVSS

SEQ ID NO: 123 - DNA, 24 bp, Artificial Sequence
  Synthetic
ggattcacccttaacaactttgtc

SEQ ID NO: 124 - protein, 8 aa, Artificial Sequence
  Synthetic
GFTLNNFV

SEQ ID NO: 125 - DNA, 24 bp, Artificial Sequence
  Synthetic
attagtgctagtggtggtagtata

SEQ ID NO: 126 - protein, 8 aa, Artificial Sequence
  Synthetic
ISASGGSI

SEQ ID NO: 127 - DNA, 36 bp, Artificial Sequence
  Synthetic
gcgaaatccccgtataactggaacccctttgactat

SEQ ID NO: 128 - protein, 12 aa, Artificial Sequence
  Synthetic
AKSPYNWNPFDY

SEQ ID NO: 129 - DNA, 327 bp, Artificial Sequence
  Synthetic
gacatccagttgacccagtctccagccaccctgtctgtgtctccaggggaacgagccaccctctcctgcagggccagtctgagtgttagcagcaaattagcctggtaccagcagacacctggccaggctcccagactcctcatctatagtgcctccacccgggccactggtatcccagtcaggttcagtggcagtgggtctgggacagagttcactctcaccatcagcagcctgcagtctgaagattttgcggtttattactgtcagcagtataatcattggcctccgtacacttttggccaggggaccaaggtggagatcaaacga

SEQ ID NO: 130 - protein, 109 aa, Artificial Sequence
  Synthetic
DIQLTQSPATLSVSPGERATLSCRASLSVSSKLAWYQQTPGQAPRLLIYSASTRATGIPVRFSGSGSGTEFTLTISSLQSEDFAVYYCQQYNHWPPYTFGQGTKVEIKR

SEQ ID NO: 131 - DNA, 18 bp, Artificial Sequence
  Synthetic
ctgagtgttagcagcaaa

SEQ ID NO: 132 - protein, 6 aa, Artificial Sequence
  Synthetic
LSVSSK

SEQ ID NO: 133 - DNA, 9 bp, Artificial Sequence
  Synthetic
agtgcctcc

SEQ ID NO: 134 - protein, 3 aa, Artificial Sequence
  Synthetic
SAS

SEQ ID NO: 135 - DNA, 30 bp, Artificial Sequence
  Synthetic
cagcagtataatcattggcctccgtacact

SEQ ID NO: 136 - protein, 10 aa, Artificial Sequence
  Synthetic
QQYNHWPPYT

SEQ ID NO: 137 - DNA, 357 bp, Artificial Sequence
  Synthetic
gaggtgcagctggtggagtctgggggaggcttggtacagcctggggggtccctgagactctcctgtgtagcttctggattcacccttaacaactttgtcatgaactgggtccgccaggttccagggaagggactggagtgggtctcttttattagtgctagtggtggtagtatatactacgcagactccgtgaagggccggttcaccatctccagagacacttccaagaacacattatatctgcaaatgaacagcctgagagccgacgacacggccgtctattactgtgcgaaatccccgtataactggaacccctttgactattggggccagggaaccctggtcaccgtctcctca

SEQ ID NO: 138 - protein, 119 aa, Artificial Sequence
  Synthetic
EVQLVESGGGLVQPGGSLRLSCVASGFTLNNFVMNWVRQVPGKGLEWVSFISASGGSIYYADSVKGRFTISRDTSKNTLYLQMNSLRADDTAVYYCAKSPYNWNPFDYWGQGTLVTVSS

SEQ ID NO: 139 - DNA, 324 bp, Artificial Sequence
  Synthetic
gaaatagtgatgacgcagtctccagccaccctgtctgtgtctccaggggaacgagccaccctctcctgcagggccagtctgagtgttagcagcaaattagcctggtaccagcagacacctggccaggctcccagactcctcatctatagtgcctccacccgggccactggtatcccagtcaggttcagtggcagtgggtctgggacagagttcactctcaccatcagcagcctgcagtctgaagattttgcggtttattactgtcagcagtataatcattggcctccgtacacttttggccaggggaccaagctggagatcaaa

SEQ ID NO: 140 - protein, 108 aa, Artificial Sequence
  Synthetic
EIVMTQSPATLSVSPGERATLSCRASLSVSSKLAWYQQTPGQAPRLLIYSASTRATGIPVRFSGSGSGTEFTLTISSLQSEDFAVYYCQQYNHWPPYTFGQGTKLEIK

SEQ ID NO: 141 - DNA, 357 bp, Artificial Sequence
  Synthetic
gaggtgcagctggtggagtctgggggaggcttggtacagcctggggggtccctgagactctcctgtgcagcctctggattcacccttaacaactttgtcatgagctgggtccgccaggctccagggaaggggctggagtgggtctcagctattagtgctagtggtggtagtatatactacgcagactccgtgaagggccggttcaccatctccagagacaattccaagaacacgctgtatctgcaaatgaacagcctgagagccgaggacacggccgtatattactgtgcgaaatccccgtataactggaacccctttgactattggggccagggaaccctggtcaccgtctcctca

SEQ ID NO: 142 - protein, 119 aa, Artificial Sequence
  Synthetic
EVQLVESGGGLVQPGGSLRLSCAASGFTLNNFVMSWVRQAPGKGLEWVSAISASGGSIYYADSVKGRFTISRDNSKNTLYLQMNSLRAEDTAVYYCAKSPYNWNPFDYWGQGTLVTVSS

SEQ ID NO: 143 - DNA, 325 bp, Artificial Sequence
  Synthetic
gaaatagtgatgacgcagtctccagccaccctgtctgtgtctccaggggaaagagccaccctctcctgcagggccagtctgagtgttagcagcaaattagcctggtaccagcagaaacctggccaggctcccaggctcctcatctatagtgcctccaccagggccactggtatcccagccaggttcagtggcagtgggtctgggacagagttcactctcaccatcagcagcctgcagtctgaagattttgcagtttattactgtcagcagtataatcattggcctccgtacacttttggccaggggaccaagctggagatcaaac

SEQ ID NO: 144 - protein, 108 aa, Artificial Sequence
  Synthetic
EIVMTQSPATLSVSPGERATLSCRASLSVSSKLAWYQQKPGQAPRLLIYSASTRATGIPARFSGSGSGTEFTLTISSLQSEDFAVYYCQQYNHWPPYTFGQGTKLEIK

SEQ ID NO: 145 - DNA, 375 bp, Artificial Sequence
  Synthetic
caggtgcagctggtggagtctgggggaggcttggaacagccgggggggtccctgagactctcctgtgcaggctctggattcacctttagagactatgccatgacctgggtccgccaggctccagggaagggactggagtgggtctcatctattagtggttccggtggtaacacatactacgcagactccgtgaagggccggttcaccatctccagagacaattccaagaacacgctgtatctgcaaatgaacagcctgagagccgaggacacggccgtatattactgtgcgaaagatcgactctctataacaattcgcccacgctattatggtttggacgtctggggccaagggtccacggtcaccgtctcctca

SEQ ID NO: 146 - protein, 125 aa, Artificial Sequence
  Synthetic
QVQLVESGGGLEQPGGSLRLSCAGSGFTFRDYAMTWVRQAPGKGLEWVSSISGSGGNTYYADSVKGRFTISRDNSKNTLYLQMNSLRAEDTAVYYCAKDRLSITIRPRYYGLDVWGQGSTVTVSS

SEQ ID NO: 147 - DNA, 24 bp, Artificial Sequence
  Synthetic
ggattcacctttagagactatgcc

SEQ ID NO: 148 - protein, 8 aa, Artificial Sequence
  Synthetic
GFTFRDYA

SEQ ID NO: 149 - DNA, 24 bp, Artificial Sequence
  Synthetic
attagtggttccggtggtaacaca

SEQ ID NO: 150 - protein, 8 aa, Artificial Sequence
  Synthetic
ISGSGGNT

SEQ ID NO: 151 - DNA, 54 bp, Artificial Sequence; identical to SEQ ID NO: 55
  Synthetic

SEQ ID NO: 152 - protein, 18 aa, Artificial Sequence
  Synthetic
AKDRLSITIRPRYYGLDV

SEQ ID NO: 153 - DNA, 339 bp, Artificial Sequence
  Synthetic
gacatcgtgttgacccagtctccactctccctgcccgtcacccctggagagccggcctccatctcctgcaggtctagtcagagcctcctgtatagtattggatacaactatttggattggtacctgcagaagtcagggcagtctccacagctccttatctatttgggttctaatcgggcctccggggtccctgacaggttcagtggcagtggatcaggcacagattttacactgaaaatcagcagagtggaggctgaggatgttgggttttattactgcatgcaagctctacaaactccgtacacttttggccaggggaccaagctggagatcaaacga

SEQ ID NO: 154 - protein, 113 aa, Artificial Sequence
  Synthetic
DIVLTQSPLSLPVTPGEPASISCRSSQSLLYSIGYNYLDWYLQKSGQSPQLLIYLGSNRASGVPDRFSGSGSGTDFTLKISRVEAEDVGFYYCMQALQTPYTFGQGTKLEIKR

SEQ ID NO: 155 - DNA, 33 bp, Artificial Sequence; identical to SEQ ID NO: 83
  Synthetic

SEQ ID NO: 156 - protein, 11 aa, Artificial Sequence
  Synthetic
QSLLYSIGYNY

SEQ ID NO: 157 - DNA, 9 bp, Artificial Sequence
  Synthetic
ttgggttct

SEQ ID NO: 158 - protein, 3 aa, Artificial Sequence
  Synthetic
LGS

SEQ ID NO: 159 - DNA, 27 bp, Artificial Sequence
  Synthetic
atgcaagctctacaaactccgtacact

SEQ ID NO: 160 - protein, 9 aa, Artificial Sequence
  Synthetic
MQALQTPYT

SEQ ID NO: 161 - DNA, 372 bp, Artificial Sequence
  Synthetic
gaggtgcagctggtggagtctgggggaggcttggaacagccgggggggtccctgagactctcctgtgcaggctctggattcacctttagagactatgccatgacctgggtccgccaggctccagggaagggactggagtgggtctcatctattagtggttccggtggtaacacatactacgcagactccgtgaagggccggttcaccatctccagagacaattccaagaacacgctgtatctgcaaatgaacagcctgagagccgaggacacggccgtatattactgtgcgaaagatcgactctctataacaattcgcccacgctattatggtttggacgtctggggccaagggaccacggtcaccgtctcc

SEQ ID NO: 162 - protein, 124 aa, Artificial Sequence
  Synthetic
EVQLVESGGGLEQPGGSLRLSCAGSGFTFRDYAMTWVRQAPGKGLEWVSSISGSGGNTYYADSVKGRFTISRDNSKNTLYLQMNSLRAEDTAVYYCAKDRLSITIRPRYYGLDVWGQGTTVTVS

SEQ ID NO: 163 - DNA, 336 bp, Artificial Sequence
  Synthetic
gacatcgtgatgacccagtctccactctccctgcccgtcacccctggagagccggcctccatctcctgcaggtctagtcagagcctcctgtatagtattggatacaactatttggattggtacctgcagaagtcagggcagtctccacagctccttatctatttgggttctaatcgggcctccggggtccctgacaggttcagtggcagtggatcaggcacagattttacactgaaaatcagcagagtggaggctgaggatgttgggttttattactgcatgcaagctctacaaactccgtacacttttggccaggggaccaagctggagatcaaa

SEQ ID NO: 164 - protein, 112 aa, Artificial Sequence [sequence omitted]

SEQ ID NO: 165 - DNA, 373 bp, Artificial Sequence
  Synthetic
gaggtgcagctggtggagtctgggggaggcttggtacagcctggggggtccctgagactctcctgtgcagcctctggattcacctttagagactatgccatgagctgggtccgccaggctccagggaaggggctggagtgggtctcagctattagtggttccggtggtaacacatactacgcagactccgtgaagggccggttcaccatctccagagacaattccaagaacacgctgtatctgcaaatgaacagcctgagagccgaggacacggccgtatattactgtgcgaaagatcgactctctataacaattcgcccacgctattatggtttggacgtctggggccaagggaccacggtcaccgtctcct

SEQ ID NO: 166 - protein, 124 aa, Artificial Sequence; identical to SEQ ID NO: 70
  Synthetic

SEQ ID NO: 167 - DNA, 337 bp, Artificial Sequence; identical to SEQ ID NO: 95
  Synthetic

SEQ ID NO: 168 - protein, 112 aa, Artificial Sequence; identical to SEQ ID NO: 96
  Synthetic

SEQ ID NO: 169 - DNA, 375 bp, Artificial Sequence
  Synthetic
caggtgcagctggtggagtctgggggagtcttggagcagcctggggggtccctgagactctcctgtacagcctctggattcacctttagagactatgccatgacctgggtccgccaggctccagggaaggggctggagtgggtctcatctattagtggtagtggtggtaatacatactacgcagactccgtgaggggccggttcaccatctccagagacaactccaaccacacgctgtatctgcaaatgaacagcctgagagccgaagacacggccgtatattactgtgcgaaagatcgactctccataacaattcgcccacgctattacggtttggacgtctggggccaagggtccacggtcaccgtctcctca

SEQ ID NO: 170 - protein, 125 aa, Artificial Sequence
  Synthetic
QVQLVESGGVLEQPGGSLRLSCTASGFTFRDYAMTWVRQAPGKGLEWVSSISGSGGNTYYADSVRGRFTISRDNSNHTLYLQMNSLRAEDTAVYYCAKDRLSITIRPRYYGLDVWGQGSTVTVSS

SEQ ID NO: 171 - DNA, 24 bp, Artificial Sequence
  Synthetic
ggattcacctttagagactatgcc

SEQ ID NO: 172 - protein, 8 aa, Artificial Sequence
  Synthetic
GFTFRDYA

SEQ ID NO: 173 - DNA, 24 bp, Artificial Sequence
  Synthetic
attagtggtagtggtggtaataca

SEQ ID NO: 174 - protein, 8 aa, Artificial Sequence
  Synthetic
ISGSGGNT

SEQ ID NO: 175 - DNA, 54 bp, Artificial Sequence
  Synthetic
gcgaaagatcgactctccataacaattcgcccacgctattacggtttggacgtc

SEQ ID NO: 176 - protein, 18 aa, Artificial Sequence
  Synthetic
AKDRLSITIRPRYYGLDV

SEQ ID NO: 177 - DNA, 324 bp, Artificial Sequence
  Synthetic
gatattgtgatgacccagtctccatcctccctgtctgcatctgtaggagacagagtcaccattacttgccgggcgagtcaggacattagcaattattttgcctggtatcagcagaagccagggaaagttcctaaactcctgatctttgctgcatccactttgcatccaggggtcccatctcggttcagtggcagtggatctgggacagatttcactctcaccattagtagcctgcagcctgaagatgttgcaacttattactgtcaaaagtataacagtgccccgtacacttttggccaggggaccaaggtggaaatcaaacga

SEQ ID NO: 178 - protein, 108 aa, Artificial Sequence
  Synthetic
DIVMTQSPSSLSASVGDRVTITCRASQDISNYFAWYQQKPGKVPKLLIFAASTLHPGVPSRFSGSGSGTDFTLTISSLQPEDVATYYCQKYNSAPYTFGQGTKVEIKR

SEQ ID NO: 179 - DNA, 18 bp, Artificial Sequence
  Synthetic
caggacattagcaattat

SEQ ID NO: 180 - protein, 6 aa, Artificial Sequence
  Synthetic
QDISNY

SEQ ID NO: 181 - DNA, 9 bp, Artificial Sequence
  Synthetic
gctgcatcc

SEQ ID NO: 182 - protein, 3 aa, Artificial Sequence
  Synthetic
AAS

SEQ ID NO: 183 - DNA, 27 bp, Artificial Sequence
  Synthetic
caaaagtataacagtgccccgtacact

SEQ ID NO: 184 - protein, 9 aa, Artificial Sequence
  Synthetic
QKYNSAPYT

SEQ ID NO: 185 - DNA, 372 bp, Artificial Sequence
  Synthetic
gaggtgcagctggtggagtctgggggagtcttggagcagcctggggggtccctgagactctcctgtacagcctctggattcacctttagagactatgccatgacctgggtccgccaggctccagggaaggggctggagtgggtctcatctattagtggtagtggtggtaatacatactacgcagactccgtgaggggccggttcaccatctccagagacaactccaaccacacgctgtatctgcaaatgaacagcctgagagccgaagacacggccgtatattactgtgcgaaagatcgactctccataacaattcgcccacgctattacggtttggacgtctggggccaagggaccacggtcaccgtctcc

SEQ ID NO: 186 - protein, 124 aa, Artificial Sequence
  Synthetic
EVQLVESGGVLEQPGGSLRLSCTASGFTFRDYAMTWVRQAPGKGLEWVSSISGSGGNTYYADSVRGRFTISRDNSNHTLYLQMNSLRAEDTAVYYCAKDRLSITIRPRYYGLDVWGQGTTVTVS

SEQ ID NO: 187 - DNA, 321 bp, Artificial Sequence
  Synthetic
gacatccagatgacccagtctccatcctccctgtctgcatctgtaggagacagagtcaccattacttgccgggcgagtcaggacattagcaattattttgcctggtatcagcagaagccagggaaagttcctaaactcctgatctttgctgcatccactttgcatccaggggtcccatctcggttcagtggcagtggatctgggacagatttcactctcaccattagtagcctgcagcctgaagatgttgcaacttattactgtcaaaagtataacagtgccccgtacacttttggccaggggaccaagctggagatcaaa

SEQ ID NO: 188 - protein, 107 aa, Artificial Sequence
  Synthetic
DIQMTQSPSSLSASVGDRVTITCRASQDISNYFAWYQQKPGKVPKLLIFAASTLHPGVPSRFSGSGSGTDFTLTISSLQPEDVATYYCQKYNSAPYTFGQGTKLEIK

SEQ ID NO: 189 - DNA, 373 bp, Artificial Sequence
  Synthetic
gaggtgcagctggtggagtctgggggaggcttggtacagcctggggggtccctgagactctcctgtgcagcctctggattcacctttagagactatgccatgagctgggtccgccaggctccagggaaggggctggagtgggtctcagctattagtggtagtggtggtaatacatactacgcagactccgtgaagggccggttcaccatctccagagacaattccaagaacacgctgtatctgcaaatgaacagcctgagagccgaggacacggccgtatattactgtgcgaaagatcgactctccataacaattcgcccacgctattacggtttggacgtctggggccaagggaccacggtcaccgtctcct

SEQ ID NO: 190 - protein, 124 aa, Artificial Sequence; identical to SEQ ID NO: 70
  Synthetic

SEQ ID NO: 191 - DNA, 322 bp, Artificial Sequence
  Synthetic
gacatccagatgacccagtctccatcctccctgtctgcatctgtaggagacagagtcaccatcacttgccgggcgagtcaggacattagcaattatttagcctggtatcagcagaaaccagggaaagttcctaagctcctgatctatgctgcatccactttgcaatcaggggtcccatctcggttcagtggcagtggatctgggacagatttcactctcaccatcagcagcctgcagcctgaagatgttgcaacttattactgtcaaaagtataacagtgccccgtacacttttggccaggggaccaagctggagatcaaac

SEQ ID NO: 192 - protein, 107 aa, Artificial Sequence
  Synthetic
DIQMTQSPSSLSASVGDRVTITCRASQDISNYLAWYQQKPGKVPKLLIYAASTLQSGVPSRFSGSGSGTDFTLTISSLQPEDVATYYCQKYNSAPYTFGQGTKLEIK

SEQ ID NO: 193 - DNA, 355 bp, Artificial Sequence
  Synthetic
gaagtgcacctggtggaatctgggggaggcttggtacagcctggcaggtccctgagactctcctgtgaggcctctggattcacctttgatgattatgccatgcactgggtccggcaagctccggggaagggcctggaatgggtctcaggtcttagtcggacaagtgtcagtataggctatgcggactctgtgaagggccgattcaccatctccagagacaacgccaagaactccctttatttggaaatgaacagtctgagacctgaggacacggccttatattactgtgcaaaatgggggacccgggggtattttgactactggggccagggaaccctggtcaccgtctcctcag

SEQ ID NO: 194 - protein, 118 aa, Artificial Sequence
  Synthetic
EVHLVESGGGLVQPGRSLRLSCEASGFTFDDYAMHWVRQAPGKGLEWVSGLSRTSVSIGYADSVKGRFTISRDNAKNSLYLEMNSLRPEDTALYYCAKWGTRGYFDYWGQGTLVTVSS

SEQ ID NO: 195 - DNA, 24 bp, Artificial Sequence
  Synthetic
ggattcacctttgatgattatgcc

SEQ ID NO: 196 - protein, 8 aa, Artificial Sequence
  Synthetic
GFTFDDYA

SEQ ID NO: 197 - DNA, 24 bp, Artificial Sequence
  Synthetic
cttagtcggacaagtgtcagtata

SEQ ID NO: 198 - protein, 8 aa, Artificial Sequence
  Synthetic
LSRTSVSI

SEQ ID NO: 199 - DNA, 33 bp, Artificial Sequence
  Synthetic
gcaaaatgggggacccgggggtattttgactac

SEQ ID NO: 200 - protein, 11 aa, Artificial Sequence
  Synthetic
AKWGTRGYFDY

SEQ ID NO: 201 - DNA, 322 bp, Artificial Sequence
  Synthetic
gacatccagatgacccagtctccatcttccgtgtctgcatctgtgggagacagagtcaccatcacttgtcgggcgagtcaggatattagtatttggttagcctggtatcagcagagtccagggaaagcccctaaactcctgatcaatgttgcatcccgtttgcaaagtggggtcccatcaaggttcagcggcagtggatctgggacagatttcactctcaccatcaacagtctgcagcctgaagattttgtaacttactattgtcaacaggctaacagtttcccgatcaccttcggccaagggacacgactggcgaccaaac

SEQ ID NO: 202 - protein, 107 aa, Artificial Sequence
  Synthetic
DIQMTQSPSSVSASVGDRVTITCRASQDISIWLAWYQQSPGKAPKLLINVASRLQSGVPSRFSGSGSGTDFTLTINSLQPEDFVTYYCQQANSFPITFGQGTRLATK

SEQ ID NO: 203 - DNA, 18 bp, Artificial Sequence
  Synthetic
caggatattagtatttgg

SEQ ID NO: 204 - protein, 6 aa, Artificial Sequence
  Synthetic
QDISIW

SEQ ID NO: 205 - DNA, 9 bp, Artificial Sequence
  Synthetic
gttgcatcc

SEQ ID NO: 206 - protein, 3 aa, Artificial Sequence
  Synthetic
VAS

SEQ ID NO: 207 - DNA, 27 bp, Artificial Sequence
  Synthetic
caacaggctaacagtttcccgatcacc

SEQ ID NO: 208 - protein, 9 aa, Artificial Sequence
  Synthetic
QQANSFPIT

SEQ ID NO: 209 - DNA, 355 bp, Artificial Sequence
  Synthetic
gaggtgcagctggtggagtctgggggaggcttggtacagcctggcaggtccctgagactctcctgtgaggcctctggattcacctttgatgattatgccatgcactgggtccggcaagctccggggaagggcctggaatgggtctcaggtcttagtcggacaagtgtcagtataggctatgcggactctgtgaagggccgattcaccatctccagagacaacgccaagaactccctttatttggaaatgaacagtctgagacctgaggacacggccttatattactgtgcaaaatgggggacccgggggtattttgactactggggccagggaaccctggtcaccgtctcctcag

SEQ ID NO: 210 - protein, 118 aa, Artificial Sequence
  Synthetic
EVQLVESGGGLVQPGRSLRLSCEASGFTFDDYAMHWVRQAPGKGLEWVSGLSRTSVSIGYADSVKGRFTISRDNAKNSLYLEMNSLRPEDTALYYCAKWGTRGYFDYWGQGTLVTVSS

SEQ ID NO: 211 - DNA, 322 bp, Artificial Sequence
  Synthetic
gacatccagatgacccagtctccatcttccgtgtctgcatctgtgggagacagagtcaccatcacttgtcgggcgagtcaggatattagtatttggttagcctggtatcagcagagtccagggaaagcccctaaactcctgatcaatgttgcatcccgtttgcaaagtggggtcccatcaaggttcagcggcagtggatctgggacagatttcactctcaccatcaacagtctgcagcctgaagattttgtaacttactattgtcaacaggctaacagtttcccgatcaccttcggccaagggacacgactggagattaaac

SEQ ID NO: 212 - protein, 107 aa, Artificial Sequence
  Synthetic
DIQMTQSPSSVSASVGDRVTITCRASQDISIWLAWYQQSPGKAPKLLINVASRLQSGVPSRFSGSGSGTDFTLTINSLQPEDFVTYYCQQANSFPITFGQGTRLEIK

SEQ ID NO: 213 - DNA, 355 bp, Artificial Sequence
  Synthetic
gaagtgcagctggtggagtctgggggaggcttggtacagcctggcaggtccctgagactctcctgtgcagcctctggattcacctttgatgattatgccatgcactgggtccggcaagctccagggaagggcctggagtgggtctcaggtcttagtcggacaagtgtcagtataggctatgcggactctgtgaagggccgattcaccatctccagagacaacgccaagaactccctgtatctgcaaatgaacagtctgagagctgaggacacggccttgtattactgtgcaaaatgggggacccgggggtattttgactactggggccaaggaaccctggtcaccgtctcctcag

SEQ ID NO: 214 - protein, 118 aa, Artificial Sequence
  Synthetic
EVQLVESGGGLVQPGRSLRLSCAASGFTFDDYAMHWVRQAPGKGLEWVSGLSRTSVSIGYADSVKGRFTISRDNAKNSLYLQMNSLRAEDTALYYCAKWGTRGYFDYWGQGTLVTVSS

SEQ ID NO: 215 - DNA, 322 bp, Artificial Sequence
  Synthetic
gacatccagatgacccagtctccatcttccgtgtctgcatctgtaggagacagagtcaccatcacttgtcgggcgagtcaggatattagtatttggttagcctggtatcagcagaaaccagggaaagcccctaagctcctgatctatgttgcatccagtttgcaaagtggggtcccatcaaggttcagcggcagtggatctgggacagatttcactctcaccatcagcagcctgcagcctgaagattttgcaacttactattgtcaacaggctaacagtttcccgatcaccttcggccaagggacacgactggagattaaac

SEQ ID NO: 216 - protein, 107 aa, Artificial Sequence
  Synthetic
DIQMTQSPSSVSASVGDRVTITCRASQDISIWLAWYQQKPGKAPKLLIYVASSLQSGVPSRFSGSGSGTDFTLTISSLQPEDFATYYCQQANSFPITFGQGTRLEIK

SEQ ID NO: 217 - DNA, 363 bp, Artificial Sequence
  Synthetic
gaggtgcagctgttggagtctgggggaggcttgctacagccgggggggtccctgagactctcctgtgcagcctctggaatcacctttagcacctatgccatgagctgggtccgtcaggctccagggagggggctggagtgggtctcagctattagtggtagtggtgatagcacatcctacgcagactccgtgaagggccggttcaccagctccagagacaattccaagaacacgctgtatctgcaaatgaacagcctgagagccgaggacacggccgtatattactgtgcgaaagtcatagcagctcgtcctcactggaacttcgatctctggggccgtggcaccctggtcactgtctcctca

SEQ ID NO: 218 - protein, 121 aa, Artificial Sequence
  Synthetic
EVQLLESGGGLLQPGGSLRLSCAASGITFSTYAMSWVRQAPGRGLEWVSAISGSGDSTSYADSVKGRFTSSRDNSKNTLYLQMNSLRAEDTAVYYCAKVIAARPHWNFDLWGRGTLVTVSS

SEQ ID NO: 219 - DNA, 24 bp, Artificial Sequence
  Synthetic
ggaatcacctttagcacctatgcc

SEQ ID NO: 220 - protein, 8 aa, Artificial Sequence
  Synthetic
GITFSTYA

SEQ ID NO: 221 - DNA, 24 bp, Artificial Sequence
  Synthetic
attagtggtagtggtgatagcaca

SEQ ID NO: 222 - protein, 8 aa, Artificial Sequence
  Synthetic
ISGSGDST

SEQ ID NO: 223 - DNA, 42 bp, Artificial Sequence
  Synthetic
gcgaaagtcatagcagctcgtcctcactggaacttcgatctc

SEQ ID NO: 224 - protein, 14 aa, Artificial Sequence
  Synthetic
AKVIAARPHWNFDL

SEQ ID NO: 225 - DNA, 324 bp, Artificial Sequence
  Synthetic
gaaattgtgttgacacagtctccagccaccctgtctttgtctccaggggaaagagccaccctctcctgcagggccagtcagagtgttagtagatatttagcctggtatcaacagaaacctggccaggctcccaggctcctcatctatgatgcatccaacagggccactggcatcccagccaggttcagtggcagtgggtctgggacagacttcactctcaccatcagcagcctagagcctgaagattttggagtttattactgtcagcagcgtagtgactggccgctcactttcggcggagggaccaaggtggagatcaaacgg

SEQ ID NO: 226 - protein, 107 aa, Artificial Sequence
  Synthetic
EIVLTQSPATLSLSPGERATLSCRASQSVSRYLAWYQQKPGQAPRLLIYDASNRATGIPARFSGSGSGTDFTLTISSLEPEDFGVYYCQQRSDWPLTFGGGTKVEIK

SEQ ID NO: 227 - DNA, 18 bp, Artificial Sequence
  Synthetic
cagagtgttagtagatat

SEQ ID NO: 228 - protein, 6 aa, Artificial Sequence
  Synthetic
QSVSRY

SEQ ID NO: 229 - DNA, 9 bp, Artificial Sequence
  Synthetic
gatgcatcc

SEQ ID NO: 230 - protein, 3 aa, Artificial Sequence
  Synthetic
DAS

SEQ ID NO: 231 - DNA, 27 bp, Artificial Sequence
  Synthetic
cagcagcgtagtgactggccgctcact

SEQ ID NO: 232 - protein, 9 aa, Artificial Sequence
  Synthetic
QQRSDWPLT

SEQ ID NO: 233 - DNA, 363 bp, Artificial Sequence; identical to SEQ ID NO: 217
  Synthetic

SEQ ID NO: 234 - protein, 121 aa, Artificial Sequence; identical to SEQ ID NO: 218
  Synthetic

SEQ ID NO: 235 - DNA, 324 bp, Artificial Sequence; identical to SEQ ID NO: 225
  Synthetic

SEQ ID NO: 236 - protein, 107 aa, Artificial Sequence; identical to SEQ ID NO: 226
  Synthetic

SEQ ID NO: 237 - DNA, 363 bp, Artificial Sequence
  Synthetic
gaggtgcagctgttggagtctgggggaggcttggtacagccgggggggtccctgagactctcctgtgcagcctctggaatcacctttagcacctatgccatgagctgggtccgtcaggctccagggaaggggctggagtgggtctcagctattagtggtagtggtgatagcacatactacgcagactccgtgaagggccggttcaccatctccagagacaattccaagaacacgctgtatctgcaaatgaacagcctgagagccgaggacacggccgtatattactgtgcgaaagtcatagcagctcgtcctcactggaacttcgatctctggggccgtggcaccctggtcactgtctcctca

SEQ ID NO: 238 - protein, 121 aa, Artificial Sequence
  Synthetic
EVQLLESGGGLVQPGGSLRLSCAASGITFSTYAMSWVRQAPGKGLEWVSAISGSGDSTYYADSVKGRFTISRDNSKNTLYLQMNSLRAEDTAVYYCAKVIAARPHWNFDLWGRGTLVTVSS

SEQ ID NO: 239 - DNA, 324 bp, Artificial Sequence
  Synthetic
gaaattgtgttgacacagtctccagccaccctgtctttgtctccaggggaaagagccaccctctcctgcagggccagtcagagtgttagtagatatttagcctggtatcaacagaaacctggccaggctcccaggctcctcatctatgatgcatccaacagggccactggcatcccagccaggttcagtggcagtgggtctgggacagacttcactctcaccatcagcagcctagagcctgaagattttgcagtttattactgtcagcagcgtagtgactggccgctcactttcggcggagggaccaaggtggagatcaaacgg

SEQ ID NO: 240 - protein, 108 aa, Artificial Sequence
  Synthetic
EIVLTQSPATLSLSPGERATLSCRASQSVSRYLAWYQQKPGQAPRLLIYDASNRATGIPARFSGSGSGTDFTLTISSLEPEDFAVYYCQQRSDWPLTFGGGTKVEIKR

SEQ ID NO: 241 - DNA, 366 bp, Artificial Sequence
  Synthetic
caggtgcagctggtggagtctgggggaggcgtggtccagcctgggaggtccctgagactcacctgtgcagcctctggattcaccttcagtagtaatggcatgcactgggtccgccaggctccaggcaaggggctggagtgggtggcaattatatcatatgatggaaataatcaatactatgcagactccgtgaagggccgattcaccatctccagagacaattccaagcacacgctgtatctggaaatgaacagcctgagagctgaggacacggctgtgtattactgtacaaaagccatctctataagtggaacttacaactggttcgattcctggggccagggaaccctggtcaccgtctcctca

SEQ ID NO: 242 - protein, 122 aa, Artificial Sequence
  Synthetic
QVQLVESGGGVVQPGRSLRLTCAASGFTFSSNGMHWVRQAPGKGLEWVAIISYDGNNQYYADSVKGRFTISRDNSKHTLYLEMNSLRAEDTAVYYCTKAISISGTYNWFDSWGQGTLVTVSS

SEQ ID NO: 243 - DNA, 24 bp, Artificial Sequence
  Synthetic
ggattcaccttcagtagtaatggc

SEQ ID NO: 244 - protein, 8 aa, Artificial Sequence
  Synthetic
GFTFSSNG

SEQ ID NO: 245 - DNA, 24 bp, Artificial Sequence
  Synthetic
atatcatatgatggaaataatcaa

SEQ ID NO: 246 - protein, 8 aa, Artificial Sequence
  Synthetic
ISYDGNNQ

SEQ ID NO: 247 - DNA, 45 bp, Artificial Sequence
  Synthetic
acaaaagccatctctataagtggaacttacaactggttcgattcc

SEQ ID NO: 248 - protein, 15 aa, Artificial Sequence
  Synthetic
TKAISISGTYNWFDS

SEQ ID NO: 249 - DNA, 324 bp, Artificial Sequence
  Synthetic
gaaattgtattgacacagtctccagccatcctgtctttgtctccaggggaaagagccaccctctcctgcagggccagtcagagtgttagcaggtacttagcctggtaccaacagaaacctggccaggctcccaggctcctcatctatgatgcatccaacagggccactggcatcccagccaggttcagtggcagtgggtctgggacagacttcactctcaccatcagcagcctagagcctgaagattttgcagtttattactgtcaacagcgtagcaactggccgctcactttcggcggagggaccaaggtggagatcaaacgg

SEQ ID NO: 250 - protein, 107 aa, Artificial Sequence
  Synthetic
EIVLTQSPAILSLSPGERATLSCRASQSVSRYLAWYQQKPGQAPRLLIYDASNRATGIPARFSGSGSGTDFTLTISSLEPEDFAVYYCQQRSNWPLTFGGGTKVEIK

SEQ ID NO: 251 - DNA, 18 bp, Artificial Sequence
  Synthetic
cagagtgttagcaggtac

SEQ ID NO: 252 - protein, 6 aa, Artificial Sequence
  Synthetic
QSVSRY

SEQ ID NO: 253 - DNA, 9 bp, Artificial Sequence
  Synthetic
gatgcatcc

SEQ ID NO: 254 - protein, 3 aa, Artificial Sequence
  Synthetic
DAS

SEQ ID NO: 255 - DNA, 27 bp, Artificial Sequence
  Synthetic
caacagcgtagcaactggccgctcact

SEQ ID NO: 256 - protein, 9 aa, Artificial Sequence
  Synthetic
QQRSNWPLT

SEQ ID NO: 257 - DNA, 366 bp, Artificial Sequence; identical to SEQ ID NO: 241
  Synthetic

SEQ ID NO: 258 - protein, 122 aa, Artificial Sequence; identical to SEQ ID NO: 242
  Synthetic

SEQ ID NO: 259 - DNA, 324 bp, Artificial Sequence; identical to SEQ ID NO: 249
  Synthetic

SEQ ID NO: 260 - protein, 107 aa, Artificial Sequence; identical to SEQ ID NO: 250
  Synthetic

SEQ ID NO: 261 - DNA, 366 bp, Artificial Sequence
  Synthetic
caggtgcagctggtggagtctgggggaggcgtggtccagcctgggaggtccctgagactctcctgtgcagcctctggattcaccttcagtagtaatggcatgcactgggtccgccaggctccaggcaaggggctggagtgggtggcagttatatcatatgatggaaataatcaatactatgcagactccgtgaagggccgattcaccatctccagagacaattccaagaacacgctgtatctgcaaatgaacagcctgagagctgaggacacggctgtgtattactgtacaaaagccatctctataagtggaacttacaactggttcgattcctggggccagggaaccctggtcaccgtctcctca

SEQ ID NO: 262 - protein, 122 aa, Artificial Sequence
  Synthetic
QVQLVESGGGVVQPGRSLRLSCAASGFTFSSNGMHWVRQAPGKGLEWVAVISYDGNNQYYADSVKGRFTISRDNSKNTLYLQMNSLRAEDTAVYYCTKAISISGTYNWFDSWGQGTLVTVSS

SEQ ID NO: 263 - DNA, 324 bp, Artificial Sequence
  Synthetic
gaaattgtattgacacagtctccagccaccctgtctttgtctccaggggaaagagccaccctctcctgcagggccagtcagagtgttagcaggtacttagcctggtaccaacagaaacctggccaggctcccaggctcctcatctatgatgcatccaacagggccactggcatcccagccaggttcagtggcagtgggtctgggacagacttcactctcaccatcagcagcctagagcctgaagattttgcagtttattactgtcaacagcgtagcaactggccgctcactttcggcggagggaccaaggtggagatcaaacgg

SEQ ID NO: 264 - protein, 108 aa, Artificial Sequence
  Synthetic
EIVLTQSPATLSLSPGERATLSCRASQSVSRYLAWYQQKPGQAPRLLIYDASNRATGIPARFSGSGSGTDFTLTISSLEPEDFAVYYCQQRSNWPLTFGGGTKVEIKR

SEQ ID NO: 265 - protein, 8 aa, Artificial Sequence
  Synthetic
  VARIANT (1)...(8): Xaa = Any amino acid
XXXXXXXX

SEQ ID NO: 266 - protein, 8 aa, Artificial Sequence
  Synthetic
  VARIANT (1)...(8): Xaa = Any amino acid
XXXXXXXX

SEQ ID NO: 267 - protein, 18 aa, Artificial Sequence
  Synthetic
  VARIANT (1)...(18): Xaa = Any amino acid
XXXXXXXXXXXXXXXXXX

SEQ ID NO: 268 - protein, 11 aa, Artificial Sequence
  Synthetic
  VARIANT (1)...(11): Xaa = Any amino acid
XXXXXXXXXXX

SEQ ID NO: 269 - protein, 3 aa, Artificial Sequence
  Synthetic
  VARIANT (1)...(3): Xaa = Any amino acid
XXX

SEQ ID NO: 270 - protein, 9 aa, Artificial Sequence
  Synthetic
  VARIANT (1)...(9): Xaa = Any amino acid
XXXXXXXXX

SEQ ID NO: 271 - protein, 330 aa, Artificial Sequence [sequence omitted]

SEQ ID NO: 272 - protein, 327 aa, Artificial Sequence
  Synthetic
ASTKGPSVFPLAPCSRSTSESTAALGCLVKDYFPEPVTVSWNSGALTSGVHTFPAVLQSSGLYSLSSVVTVPSSSLGTKTYTCNVDHKPSNTKVDKRVESKYGPPCPSCPAPEFLGGPSVFLFPPKPKDTLMISRTPEVTCVVVDVSQEDPEVQFNWYVDGVEVHNAKTKPREEQFNSTYRVVSVLTVLHQDWLNGKEYKCKVSNKGLPSSIEKTISKAKGQPREPQVYTLPPSQEEMTKNQVSLTCLVKGFYPSDIAVEWESNGQPENNYKTTPPVLDSDGSFFLYSRLTVDKSRWQEGNVFSCSVMHEALHNHYTQKSLSLSLGK

SEQ ID NO: 273 - protein, 327 aa, Artificial Sequence
  Synthetic
ASTKGPSVFPLAPCSRSTSESTAALGCLVKDYFPEPVTVSWNSGALTSGVHTFPAVLQSSGLYSLSSVVTVPSSSLGTKTYTCNVDHKPSNTKVDKRVESKYGPPCPPCPAPEFLGGPSVFLFPPKPKDTLMISRTPEVTCVVVDVSQEDPEVQFNWYVDGVEVHNAKTKPREEQFNSTYRVVSVLTVLHQDWLNGKEYKCKVSNKGLPSSIEKTISKAKGQPREPQVYTLPPSQEEMTKNQVSLTCLVKGFYPSDIAVEWESNGQPENNYKTTPPVLDSDGSFFLYSRLTVDKSRWQEGNVFSCSVMHEALHNHYTQKSLSLSLGK

SEQ ID NO: 274 - protein, 207 aa, Homo sapiens
MKVLQEPTCVSDYMSISTCEWKMNGPTNCSTELRLLYQLVFLLSEAHTCIPENNGGAGCVCHLLMDDVVSADNYTLDLWAGQQLLWKGSFKPSEHVKPRAPGNLTVHTNVSDTLLLTWSNPYPPDNYLYNHLTYAVNIWSENDPADFRIYNVTYLEPSLRIAASTLKSGISYRARVRAWAQCYNTTWSEWSPSTKWHNSYREPFEQH

SEQ ID NO: 275 - protein, 231 aa, Macaca fasicularis
MGWLCSGLLFPVSCLVLLQVASSGSMKVLQEPTCVSDYMSISTCEWKMGGPTNCSAELRLLYQLVFQSSETHTCVPENNGGVGCVCHLLMDDVVSMDNYTLDLWAGQQLLWKGSFKPSEHVKPRAPGNLTVHTNVSDTVLLTWSNPYPPDNYLYNDLTYAVNIWSENDPAYSRIHNVTYLKPTLRIPASTLKSGISYRARVRAWAQHYNTTWSEWSPSTKWYNSYREPFEQ